European Patent Specification EP 4 294 257 B1, published November 5, 2025. Title: METHOD FOR DIAGNOSING AND TREATING PARTIAL LIPODYSTROPHY. Applicant: Regeneron Pharmaceuticals, Inc. Zheng, Wenjun Harris, Charles Musser, Bret. Application TBD. The sequence listing filed with the application follows.

SEQUENCE LISTING (114 sequences)

SEQ ID NO: 1 - DNA, 357 bp, Artificial Sequence
  synthetic
caggtgcagctggtggagtctgggggaggcgtggtccagcctgggaagtccctgagactctcctgtgtagcgtctggattcaccttcagttccgatgccatgtactgggtccgccaggctccaggcaaggggctggaatgggtggcagttatttattatgatggaaattatcaatactatgaagactccgttaagggtcgattcaccatctccagagacaattcccagaacacgctggatctgcaaatgaacagcctgagagtcgacgacacggctgtatatttctgtgcgcgtctcaactgggattactggtatctcgatctctggggccgtggcaccctggtcactgtctcctca

SEQ ID NO: 2 - protein, 119 aa, Artificial Sequence
  synthetic
QVQLVESGGGVVQPGKSLRLSCVASGFTFSSDAMYWVRQAPGKGLEWVAVIYYDGNYQYYEDSVKGRFTISRDNSQNTLDLQMNSLRVDDTAVYFCARLNWDYWYLDLWGRGTLVTVSS

SEQ ID NO: 3 - DNA, 24 bp, Artificial Sequence
  synthetic
ggattcaccttcagttccgatgcc

SEQ ID NO: 4 - protein, 8 aa, Artificial Sequence
  synthetic
GFTFSSDA

SEQ ID NO: 5 - DNA, 24 bp, Artificial Sequence
  synthetic
atttattatgatggaaattatcaa

SEQ ID NO: 6 - protein, 8 aa, Artificial Sequence
  synthetic
IYYDGNYQ

SEQ ID NO: 7 - DNA, 36 bp, Artificial Sequence
  synthetic
gcgcgtctcaactgggattactggtatctcgatctc

SEQ ID NO: 8 - protein, 12 aa, Artificial Sequence
  synthetic
ARLNWDYWYLDL

SEQ ID NO: 9 - DNA, 324 bp, Artificial Sequence
  synthetic
gacatccagatgacccagtctccatcctccctgtctgcatctgtaggagacagagtcaccatcacttgccgggcaagtcagagcattagcagctatttaaattggtatcagcagaaaccagggaaagcccctaagctcctgatctatgctgcatccagtttgcaaagtggggtcccgtcaaggttcagtggcagtggatctgggacagatttcactctcaccatcagcagtctgcaacctgaagattttgcaacttactactgtcaacagagttacagtacccctccgatcaccttcggccaagggacacgactggagattaaa

SEQ ID NO: 10 - protein, 108 aa, Artificial Sequence
  synthetic
DIQMTQSPSSLSASVGDRVTITCRASQSISSYLNWYQQKPGKAPKLLIYAASSLQSGVPSRFSGSGSGTDFTLTISSLQPEDFATYYCQQSYSTPPITFGQGTRLEIK

SEQ ID NO: 11 - DNA, 18 bp, Artificial Sequence
  synthetic
cagagcattagcagctat

SEQ ID NO: 12 - protein, 6 aa, Artificial Sequence
  synthetic
QSISSY

SEQ ID NO: 13 - DNA, 9 bp, Artificial Sequence
  synthetic
gctgcatcc

SEQ ID NO: 14 - protein, 3 aa, Artificial Sequence
  synthetic
AAS

SEQ ID NO: 15 - DNA, 30 bp, Artificial Sequence
  synthetic
caacagagttacagtacccctccgatcacc

SEQ ID NO: 16 - protein, 10 aa, Artificial Sequence
  synthetic
QQSYSTPPIT

SEQ ID NO: 17 - DNA, 357 bp, Artificial Sequence
  synthetic
caggtgcagctggtggagtccgggggaggcgtggtccagcctgggaggtccctgagactctcctgtacagcgtctggattcaccttcagtagttatgccatgtactgggtccgccaggctccaggcaaggggctggagtgggtgtcagttatatactatgatggaagttataaatactatgcagactccgtgaagggccgattcaccatctccagagacaattccaagaacacgctgtatctgcaaatggacagcctgagagccgaggacacggctgtctattactgtgcgagttataactggaactactggtacttcgatttctggggccgtggcaccctggtcactgtctcctca

SEQ ID NO: 18 - protein, 119 aa, Artificial Sequence
  synthetic
QVQLVESGGGVVQPGRSLRLSCTASGFTFSSYAMYWVRQAPGKGLEWVSVIYYDGSYKYYADSVKGRFTISRDNSKNTLYLQMDSLRAEDTAVYYCASYNWNYWYFDFWGRGTLVTVSS

SEQ ID NO: 19 - DNA, 24 bp, Artificial Sequence
  synthetic
ggattcaccttcagtagttatgcc

SEQ ID NO: 20 - protein, 8 aa, Artificial Sequence
  synthetic
GFTFSSYA

SEQ ID NO: 21 - DNA, 24 bp, Artificial Sequence
  synthetic
atatactatgatggaagttataaa

SEQ ID NO: 22 - protein, 8 aa, Artificial Sequence
  synthetic
IYYDGSYK

SEQ ID NO: 23 - DNA, 36 bp, Artificial Sequence
  synthetic
gcgagttataactggaactactggtacttcgatttc

SEQ ID NO: 24 - protein, 12 aa, Artificial Sequence
  synthetic
ASYNWNYWYFDF

SEQ ID NO: 25 - DNA, 357 bp, Artificial Sequence
  synthetic
caggtgcagctggtggagtctgggggaagcgtggtccagcctgggaggtccctgagactctcctgtgcagcgtctggattcaccttcagtacatatgccatgtactgggtccgccagactccaggcaaggggctggagtgggtggctgttttatactctgatggaagtaataaatactatatagactccgtgaagggccgattcaccatctccagagacacttccacgaacactctgtatctgcaaatgagcagcctgcgagccgacgactcggctctatattactgtgcgcgtctcaactgggattactggtacttcgatctctggggccgtggcaccctggtcactgtctcctca

SEQ ID NO: 26 - protein, 119 aa, Artificial Sequence
  synthetic
QVQLVESGGSVVQPGRSLRLSCAASGFTFSTYAMYWVRQTPGKGLEWVAVLYSDGSNKYYIDSVKGRFTISRDTSTNTLYLQMSSLRADDSALYYCARLNWDYWYFDLWGRGTLVTVSS

SEQ ID NO: 27 - DNA, 24 bp, Artificial Sequence
  synthetic
ggattcaccttcagtacatatgcc

SEQ ID NO: 28 - protein, 8 aa, Artificial Sequence
  synthetic
GFTFSTYA

SEQ ID NO: 29 - DNA, 24 bp, Artificial Sequence
  synthetic
ttatactctgatggaagtaataaa

SEQ ID NO: 30 - protein, 8 aa, Artificial Sequence
  synthetic
LYSDGSNK

SEQ ID NO: 31 - DNA, 36 bp, Artificial Sequence
  synthetic
gcgcgtctcaactgggattactggtacttcgatctc

SEQ ID NO: 32 - protein, 12 aa, Artificial Sequence
  synthetic
ARLNWDYWYFDL

SEQ ID NO: 33 - DNA, 357 bp, Artificial Sequence
  synthetic
caggtgcagctggtggagtctgggggaggcgtggtccagcctgggaggtccctgagactctcctgtgaagcgtctggattcagcagcagtgacaatgccatgtactgggtccgccaggctccaggcaaggggctggagtgggtgtcagttatatatcatgatggaagttataaatactatgaagactccgtgaagggccgattcaccatcgccagagacaattccaagaacacgctttatttgcaaatgaacagcctgagagccgaggacacggctgtatattactgtgcgaggtataactggaaccactggtacttcgatgtctggggccgtggcaccctggtcactgtctcctca

SEQ ID NO: 34 - protein, 119 aa, Artificial Sequence
  synthetic
QVQLVESGGGVVQPGRSLRLSCEASGFSSSDNAMYWVRQAPGKGLEWVSVIYHDGSYKYYEDSVKGRFTIARDNSKNTLYLQMNSLRAEDTAVYYCARYNWNHWYFDVWGRGTLVTVSS

SEQ ID NO: 35 - DNA, 24 bp, Artificial Sequence
  synthetic
ggattcagcagcagtgacaatgcc

SEQ ID NO: 36 - protein, 8 aa, Artificial Sequence
  synthetic
GFSSSDNA

SEQ ID NO: 37 - DNA, 24 bp, Artificial Sequence
  synthetic
atatatcatgatggaagttataaa

SEQ ID NO: 38 - protein, 8 aa, Artificial Sequence
  synthetic
IYHDGSYK

SEQ ID NO: 39 - DNA, 36 bp, Artificial Sequence
  synthetic
gcgaggtataactggaaccactggtacttcgatgtc

SEQ ID NO: 40 - protein, 12 aa, Artificial Sequence
  synthetic
ARYNWNHWYFDV

SEQ ID NO: 41 - DNA, 366 bp, Artificial Sequence
  synthetic
caggtgcagctggtggagtctgggggaggcgtggtccagcctgggaggtccctgagactctcctgtgcagcctctggattcaccttcagtacctatggcatgcactgggtccgccaggctccaggcaaggggctggagtgggtgtcagttatatcatatgacgaaagtaataagtactatgcagactccgtgaagggccgattcaccatttctagagacaattccaagaacgcgctgtatttacaaatgaacagcctgagaaatgaggacacggctgtgtattactgtgcgagagatcggccttttggattggttaccggatggttcgacccctggggccagggaaccctggtcaccgtctcctca

SEQ ID NO: 42 - protein, 122 aa, Artificial Sequence
  synthetic
QVQLVESGGGVVQPGRSLRLSCAASGFTFSTYGMHWVRQAPGKGLEWVSVISYDESNKYYADSVKGRFTISRDNSKNALYLQMNSLRNEDTAVYYCARDRPFGLVTGWFDPWGQGTLVTVSS

SEQ ID NO: 43 - DNA, 24 bp, Artificial Sequence
  synthetic
ggattcaccttcagtacctatggc

SEQ ID NO: 44 - protein, 8 aa, Artificial Sequence
  synthetic
GFTFSTYG

SEQ ID NO: 45 - DNA, 24 bp, Artificial Sequence
  synthetic
atatcatatgacgaaagtaataag

SEQ ID NO: 46 - protein, 8 aa, Artificial Sequence
  synthetic
ISYDESNK

SEQ ID NO: 47 - DNA, 45 bp, Artificial Sequence
  synthetic
gcgagagatcggccttttggattggttaccggatggttcgacccc

SEQ ID NO: 48 - protein, 15 aa, Artificial Sequence
  synthetic
ARDRPFGLVTGWFDP

SEQ ID NO: 49 - DNA, 360 bp, Artificial Sequence
  synthetic
caggtgcagctggtggagtctgggggaggcgtggtccagcctgggaggtccctgagactctcctgtgcagcgtctggattcagtttcaatacctatggcatgcactgggtccgccaggctccaggcaaggggctggagtgggtgacaattatatggtatgatggaagtattaaatactatgcagactccgtgaagggccgattcaccatctccagagacaattccaagaacacgctgtatctgcaaatgaacagcctgagagccgaggacacggctgtgtattattgtgcgagaggtggatatagtggctacctctactttgactactggggccagggaaccctggtcaccgtctcctca

SEQ ID NO: 50 - protein, 120 aa, Artificial Sequence
  synthetic
QVQLVESGGGVVQPGRSLRLSCAASGFSFNTYGMHWVRQAPGKGLEWVTIIWYDGSIKYYADSVKGRFTISRDNSKNTLYLQMNSLRAEDTAVYYCARGGYSGYLYFDYWGQGTLVTVSS

SEQ ID NO: 51 - DNA, 24 bp, Artificial Sequence
  synthetic
ggattcagtttcaatacctatggc

SEQ ID NO: 52 - protein, 8 aa, Artificial Sequence
  synthetic
GFSFNTYG

SEQ ID NO: 53 - DNA, 24 bp, Artificial Sequence
  synthetic
atatggtatgatggaagtattaaa

SEQ ID NO: 54 - protein, 8 aa, Artificial Sequence
  synthetic
IWYDGSIK

SEQ ID NO: 55 - DNA, 39 bp, Artificial Sequence
  synthetic
gcgagaggtggatatagtggctacctctactttgactac

SEQ ID NO: 56 - protein, 13 aa, Artificial Sequence
  synthetic
ARGGYSGYLYFDY

SEQ ID NO: 57 - DNA, 372 bp, Artificial Sequence
  synthetic
caggtgcagctgcaggagtcgggcccaggactggtgaagccttcacagaccctgtccctcacctgcactgtctctggtggctccatcagcagcggtggtgactactggagctggatccgccagctcccagggaagggcctggagtggattgggtacatctattacagtgggagcgcctactataatccgtccctcaagagtcgaggtaccatatcaatagacacgtctaagaaccagttctccctgaagctgacctctgtgactgccgcggacacggccgtatatttctgtgtgaaattacgatttttggagtggttcttggggggctggttcggcccctggggccagggaaccctggtcaccgtctcctca

SEQ ID NO: 58 - protein, 124 aa, Artificial Sequence
  synthetic
QVQLQESGPGLVKPSQTLSLTCTVSGGSISSGGDYWSWIRQLPGKGLEWIGYIYYSGSAYYNPSLKSRGTISIDTSKNQFSLKLTSVTAADTAVYFCVKLRFLEWFLGGWFGPWGQGTLVTVSS

SEQ ID NO: 59 - DNA, 30 bp, Artificial Sequence
  synthetic
ggtggctccatcagcagcggtggtgactac

SEQ ID NO: 60 - protein, 10 aa, Artificial Sequence
  synthetic
GGSISSGGDY

SEQ ID NO: 61 - DNA, 21 bp, Artificial Sequence
  synthetic
atctattacagtgggagcgcc

SEQ ID NO: 62 - protein, 7 aa, Artificial Sequence
  synthetic
IYYSGSA

SEQ ID NO: 63 - DNA, 48 bp, Artificial Sequence
  synthetic
gtgaaattacgatttttggagtggttcttggggggctggttcggcccc

SEQ ID NO: 64 - protein, 16 aa, Artificial Sequence
  synthetic
VKLRFLEWFLGGWFGP

SEQ ID NO: 65 - DNA, 351 bp, Artificial Sequence
  synthetic
gaggtgcagctggtggagtctgggggaggcttggtacagccgggggggtccctgagactctcctgtgcagcctctggattcacctttagcaactatggcatgacctgggtccgccaggctccagggaagggcctggaatgggtctcagctattactggtggtggtggtagcacatactactcaaactccgtgaagggccggttcaccatctccagagacaattccaagaacacggtgtatctgcgaatgaacagtgtgagagccgaggacacggccgtatattactgtgcgaaatataagtggaacttcgtggacgactggggccagggaaccacggtcaccgtctcctca

SEQ ID NO: 66 - protein, 117 aa, Artificial Sequence
  synthetic
EVQLVESGGGLVQPGGSLRLSCAASGFTFSNYGMTWVRQAPGKGLEWVSAITGGGGSTYYSNSVKGRFTISRDNSKNTVYLRMNSVRAEDTAVYYCAKYKWNFVDDWGQGTTVTVSS

SEQ ID NO: 67 - DNA, 24 bp, Artificial Sequence
  synthetic
ggattcacctttagcaactatggc

SEQ ID NO: 68 - protein, 8 aa, Artificial Sequence
  synthetic
GFTFSNYG

SEQ ID NO: 69 - DNA, 24 bp, Artificial Sequence
  synthetic
attactggtggtggtggtagcaca

SEQ ID NO: 70 - protein, 8 aa, Artificial Sequence
  synthetic
ITGGGGST

SEQ ID NO: 71 - DNA, 30 bp, Artificial Sequence
  synthetic
gcgaaatataagtggaacttcgtggacgac

SEQ ID NO: 72 - protein, 10 aa, Artificial Sequence
  synthetic
AKYKWNFVDD

SEQ ID NO: 73 - DNA, 360 bp, Artificial Sequence
  synthetic
gaggtgcagctggtggagtctgggggaggcttggtacagcctggggggtccctgagactctcctgtgttgcctctggattcaccttcaataaatacgacatgcactgggtccgccaaactactggaaaaggtctagagtgggtctcaggtattgatactgatggtgacacatactatccaggctccgtgaagggccgattcaccatctccagagaaaatgccgagaactccctgtatcttcaaatgaacggcctgagagtcggggacacggctgtgtattactgtgcaagatggccttggagtggtttctatggtgcttttgatatctggggccaagggacaatggtcaccgtctcttca

SEQ ID NO: 74 - protein, 120 aa, Artificial Sequence
  synthetic
EVQLVESGGGLVQPGGSLRLSCVASGFTFNKYDMHWVRQTTGKGLEWVSGIDTDGDTYYPGSVKGRFTISRENAENSLYLQMNGLRVGDTAVYYCARWPWSGFYGAFDIWGQGTMVTVSS

SEQ ID NO: 75 - DNA, 24 bp, Artificial Sequence
  synthetic
ggattcaccttcaataaatacgac

SEQ ID NO: 76 - protein, 8 aa, Artificial Sequence
  synthetic
GFTFNKYD

SEQ ID NO: 77 - DNA, 21 bp, Artificial Sequence
  synthetic
attgatactgatggtgacaca

SEQ ID NO: 78 - protein, 7 aa, Artificial Sequence
  synthetic
IDTDGDT

SEQ ID NO: 79 - DNA, 42 bp, Artificial Sequence
  synthetic
gcaagatggccttggagtggtttctatggtgcttttgatatc

SEQ ID NO: 80 - protein, 14 aa, Artificial Sequence
  synthetic
ARWPWSGFYGAFDI

SEQ ID NO: 81 - DNA, 366 bp, Artificial Sequence
  synthetic
caggtgcagctgcaggagtcgggcccaggactggtgaagccttcacagaccctgtccctcacctgcactgtctctggtggctccatcagcagtggtaattactactggaactggatccgccaacagccaggagagggcctggagtggattgcttacatctatcacaatggggtcaccaacttcaatccgtccctcaagagtcgacttactatatcagtagacacgtctaagactcagttctccctgaagttgaggtctgtgactgccgcggacacggccgtttattactgtgcgagatcaggcagctggttcgagaactggtacttcgatctctggggccgtggcaccctggtcactgtctcctca

SEQ ID NO: 82 - protein, 122 aa, Artificial Sequence
  synthetic
QVQLQESGPGLVKPSQTLSLTCTVSGGSISSGNYYWNWIRQQPGEGLEWIAYIYHNGVTNFNPSLKSRLTISVDTSKTQFSLKLRSVTAADTAVYYCARSGSWFENWYFDLWGRGTLVTVSS

SEQ ID NO: 83 - DNA, 30 bp, Artificial Sequence
  synthetic
ggtggctccatcagcagtggtaattactac

SEQ ID NO: 84 - protein, 10 aa, Artificial Sequence
  synthetic
GGSISSGNYY

SEQ ID NO: 85 - DNA, 21 bp, Artificial Sequence
  synthetic
atctatcacaatggggtcacc

SEQ ID NO: 86 - protein, 7 aa, Artificial Sequence
  synthetic
IYHNGVT

SEQ ID NO: 87 - DNA, 42 bp, Artificial Sequence
  synthetic
gcgagatcaggcagctggttcgagaactggtacttcgatctc

SEQ ID NO: 88 - protein, 14 aa, Artificial Sequence
  synthetic
ARSGSWFENWYFDL

SEQ ID NO: 89 - DNA, 324 bp, Artificial Sequence
  synthetic
gaaattgtgttgacgcagtctccaggcaccctgtctttgtctccaggggaaagagccaccctctcctgcagggccagtcagagtgttagcagcagctacttagcctggtaccagcagaaacctggccaggctcccaggctcctcatctatggtgcatccagcagggccactggcatcccagacaggttcagtggcagtgggtctgggacagacttcactctcaccatcagcagactggagcctgaagattttgcagtgtattactgtcagcagtatggtagctcaccttggacgttcggccaagggaccaaggtggaaatcaaa

SEQ ID NO: 90 - protein, 108 aa, Artificial Sequence
  synthetic
EIVLTQSPGTLSLSPGERATLSCRASQSVSSSYLAWYQQKPGQAPRLLIYGASSRATGIPDRFSGSGSGTDFTLTISRLEPEDFAVYYCQQYGSSPWTFGQGTKVEIK

SEQ ID NO: 91 - DNA, 21 bp, Artificial Sequence
  synthetic
cagagtgttagcagcagctac

SEQ ID NO: 92 - protein, 7 aa, Artificial Sequence
  synthetic
QSVSSSY

SEQ ID NO: 93 - DNA, 9 bp, Artificial Sequence
  synthetic
ggtgcatcc

SEQ ID NO: 94 - protein, 3 aa, Artificial Sequence
  synthetic
GAS

SEQ ID NO: 95 - DNA, 27 bp, Artificial Sequence
  synthetic
cagcagtatggtagctcaccttggacg

SEQ ID NO: 96 - protein, 9 aa, Artificial Sequence
  synthetic
QQYGSSPWT

SEQ ID NO: 97 - DNA, 360 bp, Artificial Sequence
  synthetic
caggtgcagctgcaggagtcgggcccaggactggtgaagccttcggagaccctgtccctcacctgcactgtctctggtggctccatcagtaattcctactggagctggatccggcagcccccagggaagggactggagtggattggatatgtctattcccgtgggaacaccaagtacaacccctccctcacgagtcgagtcaccatgtcatttgacacgtccaagaaccagttctccctgaaactgaggtctgtgaccgccgcagacacggccgtgtattactgtgcgagaagcagcagctggtacgaggactggtacttcgatctctggggccgtggcaccctggtcactgtctcctca

SEQ ID NO: 98 - protein, 120 aa, Artificial Sequence
  synthetic
QVQLQESGPGLVKPSETLSLTCTVSGGSISNSYWSWIRQPPGKGLEWIGYVYSRGNTKYNPSLTSRVTMSFDTSKNQFSLKLRSVTAADTAVYYCARSSSWYEDWYFDLWGRGTLVTVSS

SEQ ID NO: 99 - DNA, 24 bp, Artificial Sequence
  synthetic
ggtggctccatcagtaattcctac

SEQ ID NO: 100 - protein, 8 aa, Artificial Sequence
  synthetic
GGSISNSY

SEQ ID NO: 101 - DNA, 21 bp, Artificial Sequence
  synthetic
gtctattcccgtgggaacacc

SEQ ID NO: 102 - protein, 7 aa, Artificial Sequence
  synthetic
VYSRGNT

SEQ ID NO: 103 - DNA, 42 bp, Artificial Sequence
  synthetic
gcgagaagcagcagctggtacgaggactggtacttcgatctc

SEQ ID NO: 104 - protein, 14 aa, Artificial Sequence
  synthetic
ARSSSWYEDWYFDL

SEQ ID NO: 105 - DNA, 354 bp, Artificial Sequence
  synthetic
caggtgcagctacagcagtggggcgcagggctgtttaagccttcggagaccctgtccctcacctgcgatgtctatggtgggtccttcagaggttattattggagttggatccgccagcccccagggaaggggctggagtggattggggaaatcagttatagtggtttcaccaattacaacccgtccctcaagagtcgagtcatcatatcaatagatacgtccaagaaccagttctccctgaagatgagctctgtgaccgccgcggacacggctgtttattactgtgcgagagttacctatggttatgggacctttgattattggggccagggaaccctggtcaccgtctcctca

SEQ ID NO: 106 - protein, 118 aa, Artificial Sequence
  synthetic
QVQLQQWGAGLFKPSETLSLTCDVYGGSFRGYYWSWIRQPPGKGLEWIGEISYSGFTNYNPSLKSRVIISIDTSKNQFSLKMSSVTAADTAVYYCARVTYGYGTFDYWGQGTLVTVSS

SEQ ID NO: 107 - DNA, 24 bp, Artificial Sequence
  synthetic
ggtgggtccttcagaggttattat

SEQ ID NO: 108 - protein, 8 aa, Artificial Sequence
  synthetic
GGSFRGYY

SEQ ID NO: 109 - DNA, 21 bp, Artificial Sequence
  synthetic
atcagttatagtggtttcacc

SEQ ID NO: 110 - protein, 7 aa, Artificial Sequence
  synthetic
ISYSGFT

SEQ ID NO: 111 - DNA, 36 bp, Artificial Sequence
  synthetic
gcgagagttacctatggttatgggacctttgattat

SEQ ID NO: 112 - protein, 12 aa, Artificial Sequence
  synthetic
ARVTYGYGTFDY

SEQ ID NO: 113 - protein, 446 aa, Artificial Sequence
  synthetic
QVQLVESGGSVVQPGRSLRLSCAASGFTFSTYAMYWVRQTPGKGLEWVAVLYSDGSNKYYIDSVKGRFTISRDTSTNTLYLQMSSLRADDSALYYCARLNWDYWYFDLWGRGTLVTVSSASTKGPSVFPLAPCSRSTSESTAALGCLVKDYFPEPVTVSWNSGALTSGVHTFPAVLQSSGLYSLSSVVTVPSSSLGTKTYTCNVDHKPSNTKVDKRVESKYGPPCPPCPAPEFLGGPSVFLFPPKPKDTLMISRTPEVTCVVVDVSQEDPEVQFNWYVDGVEVHNAKTKPREEQFNSTYRVVSVLTVLHQDWLNGKEYKCKVSNKGLPSSIEKTISKAKGQPREPQVYTLPPSQEEMTKNQVSLTCLVKGFYPSDIAVEWESNGQPENNYKTTPPVLDSDGSFFLYSRLTVDKSRWQEGNVFSCSVMHEALHNHYTQKSLSLSLGK

SEQ ID NO: 114 - protein, 215 aa, Artificial Sequence
  synthetic
DIQMTQSPSSLSASVGDRVTITCRASQSISSYLNWYQQKPGKAPKLLIYAASSLQSGVPSRFSGSGSGTDFTLTISSLQPEDFATYYCQQSYSTPPITFGQGTRLEIKRTVAAPSVFIFPPSDEQLKSGTASVVCLLNNFYPREAKVQWKVDNALQSGNSQESVTEQDSKDSTYSLSSTLTLSKADYEKHKVYACEVTHQGLSSPVTKSFNRGEC